European Patent Specification EP 4 010 082 B1, published January 25, 2023. Title: MULTISPECIFIC ANTI-TCR DELTA VARIABLE 1 ANTIBODIES. Applicant: GammaDelta Therapeutics Limited. The sequence listing filed with the application follows.

SEQUENCE LISTING (176 sequences)

SEQ ID NO: 1 - protein, 209 aa, Homo sapiens
  Variable delta 1 (V delta 1) chain of a gamma delta T cell receptor (TCR) (human)
AQKVTQAQSSVSMPVRKAVTLNCLYETSWWSYYIFWYKQLPSKEMIFLIRQGSDEQNAKSGRYSVNFKKAAKSVALTISALQLEDSAKYFCALGESLTRADKLIFGKGTRVTVEPNIQNPDPAVYQLRDSKSSDKSVCLFTDFDSQTNVSQSKDSDVYITDKTVLDMRSMDFKSNSAVAWSNKSDFACANAFNNSIIPEDTFFPSPESS

SEQ ID NO: 2 - protein, 9 aa, Homo sapiens
  E07 Heavy CDR3
VDYADAFDI

SEQ ID NO: 3 - protein, 9 aa, Homo sapiens
  C08 Heavy CDR3
PIELGAFDI

SEQ ID NO: 4 - protein, 8 aa, Homo sapiens
  G04 Heavy CDR3
TWSGYVDV

SEQ ID NO: 5 - protein, 9 aa, Homo sapiens
  B07 Heavy CDR3
ENYLNAFDI

SEQ ID NO: 6 - protein, 8 aa, Homo sapiens
  C05 Heavy CDR3
DSGVAFDI

SEQ ID NO: 7 - protein, 10 aa, Homo sapiens
  E01 Heavy CDR3
HQVDTRTADY

SEQ ID NO: 8 - protein, 8 aa, Homo sapiens
  E04 Heavy CDR3
SWNDAFDI

SEQ ID NO: 9 - protein, 8 aa, Homo sapiens
  F07 Heavy CDR3
DYYYSMDV

SEQ ID NO: 10 - protein, 9 aa, Homo sapiens
  G06 Heavy CDR3
HSWNDAFDV

SEQ ID NO: 11 - protein, 8 aa, Homo sapiens
  G09 Heavy CDR3
DYYYSMDV

SEQ ID NO: 12 - protein, 9 aa, Homo sapiens
  B09 Heavy CDR3
HSWSDAFDI

SEQ ID NO: 13 - protein, 9 aa, Homo sapiens
  G10 Heavy CDR3
HSWNDAFDI

SEQ ID NO: 14 - protein, 9 aa, Homo sapiens
  E07 Light CDR3
QQSYSTLLT

SEQ ID NO: 15 - protein, 11 aa, Homo sapiens
  C08 Light CDR3
QVWDSSSDHVV

SEQ ID NO: 16 - protein, 10 aa, Homo sapiens
  G04 Light CDR3
QQSYSTPQVT

SEQ ID NO: 17 - protein, 9 aa, Homo sapiens
  B07 Light CDR3
QQSYSTPLT

SEQ ID NO: 18 - protein, 9 aa, Homo sapiens
  C05 Light CDR3
QQFKRYPPT

SEQ ID NO: 19 - protein, 10 aa, Homo sapiens
  E01 Light CDR3
SSYTSTSTLV

SEQ ID NO: 20 - protein, 9 aa, Homo sapiens
  E04 Light CDR3
QQSYSTPLT

SEQ ID NO: 21 - protein, 9 aa, Homo sapiens
  F07 Light CDR3
QQSHSHPPT

SEQ ID NO: 22 - protein, 9 aa, Homo sapiens
  G06 Light CDR3
QQSYSTPDT

SEQ ID NO: 23 - protein, 9 aa, Homo sapiens
  G09 Light CDR3
QQSYSTPVT

SEQ ID NO: 24 - protein, 9 aa, Homo sapiens
  B09 Light CDR3
QQSYSTPLT

SEQ ID NO: 25 - protein, 9 aa, Homo sapiens
  G10 Light CDR3
QQSYSTLLT

SEQ ID NO: 26 - protein, 8 aa, Homo sapiens
  E07 Heavy CDR2
ISSSGSTI

SEQ ID NO: 27 - protein, 7 aa, Homo sapiens
  C08 Heavy CDR2
IYSGGST

SEQ ID NO: 28 - protein, 9 aa, Homo sapiens
  G04 Heavy CDR2
TYYRSKWST

SEQ ID NO: 29 - protein, 8 aa, Homo sapiens
  G04 Heavy CDR2
ISSSGSTI

SEQ ID NO: 30 - protein, 8 aa, Homo sapiens
  C05 Heavy CDR2
ISGGGGTT

SEQ ID NO: 31 - protein, 8 aa, Homo sapiens
  E01 Heavy CDR2
IYPGDSDT

SEQ ID NO: 32 - protein, 9 aa, Homo sapiens
  E04 Heavy CDR2
TYYRSKWYN

SEQ ID NO: 33 - protein, 9 aa, Homo sapiens
  F07 Heavy CDR2
TYYRSKWYN

SEQ ID NO: 34 - protein, 8 aa, Homo sapiens
  G06 Heavy CDR2
ISSSGSTI

SEQ ID NO: 35 - protein, 9 aa, Homo sapiens
  G09 Heavy CDR2
TYYGSKWYN

SEQ ID NO: 36 - protein, 8 aa, Homo sapiens
  B09 Heavy CDR2
ISSSGSTI

SEQ ID NO: 37 - protein, 8 aa, Homo sapiens
  G10 Heavy CDR2
ISSSGSTI

SEQ ID NO: 38 - protein, 8 aa, Homo sapiens
  E07 Heavy CDR1
GFTFSDYY

SEQ ID NO: 39 - protein, 8 aa, Homo sapiens
  C08 Heavy CDR1
GFTVSSNY

SEQ ID NO: 40 - protein, 10 aa, Homo sapiens
  G04 Heavy CDR1
GDSVSSKSAA

SEQ ID NO: 41 - protein, 8 aa, Homo sapiens
  B07 Heavy CDR1
GFTFSDYY

SEQ ID NO: 42 - protein, 8 aa, Homo sapiens
  C05 Heavy CDR1
GFTFSSYA

SEQ ID NO: 43 - protein, 8 aa, Homo sapiens
  E01 Heavy CDR1
GYSFTSYW

SEQ ID NO: 44 - protein, 10 aa, Homo sapiens
  E04 Heavy CDR1
GDSVSSNSAA

SEQ ID NO: 45 - protein, 10 aa, Homo sapiens
  F07 Heavy CDR1
GDSVSSNSAA

SEQ ID NO: 46 - protein, 8 aa, Homo sapiens
  G06 Heavy CDR1
GFTFSDYY

SEQ ID NO: 47 - protein, 10 aa, Homo sapiens
  G09 Heavy CDR1
GDSVSSNSAA

SEQ ID NO: 48 - protein, 8 aa, Homo sapiens
  B09 Heavy CDR1
GFTFSDYY

SEQ ID NO: 49 - protein, 8 aa, Homo sapiens
  G10 Heavy CDR1
GFTFSDYY

SEQ ID NO: 50 - protein, 6 aa, Homo sapiens
  E07 Light CDR1
QSIGTY

SEQ ID NO: 51 - protein, 6 aa, Homo sapiens
  C08 Light CDR1
NIGSQS

SEQ ID NO: 52 - protein, 6 aa, Homo sapiens
  G04 Light CDR1
QDINDW

SEQ ID NO: 53 - protein, 6 aa, Homo sapiens
  B07 Light CDR1
QSLSNY

SEQ ID NO: 54 - protein, 6 aa, Homo sapiens
  C05 Light CDR1
QNIRTW

SEQ ID NO: 55 - protein, 9 aa, Homo sapiens
  E01 Light CDR1
RSDVGGYNY

SEQ ID NO: 56 - protein, 6 aa, Homo sapiens
  E04 Light CDR1
QSISTW

SEQ ID NO: 57 - protein, 6 aa, Homo sapiens
  F07 Light CDR1
QSISSW

SEQ ID NO: 58 - protein, 6 aa, Homo sapiens
  G06 Light CDR1
QSISSY

SEQ ID NO: 59 - protein, 6 aa, Homo sapiens
  G09 Light CDR1
QSISTW

SEQ ID NO: 60 - protein, 6 aa, Homo sapiens
  B09 Light CDR1
QDISNY

SEQ ID NO: 61 - protein, 6 aa, Homo sapiens
  G10 Light CDR1
QSISSH

SEQ ID NO: 62 - protein, 118 aa, Homo sapiens
  E07 VH region
QVQLVESGGGLVKPGGSLRLSCAASGFTFSDYYMSWIRQAPGKGLEWVSYISSSGSTIYYADSVKGRFTISRDNAKNSLYLQMNSLRAEDTAVYYCARVDYADAFDIWGQGTLVTVSS

SEQ ID NO: 63 - protein, 117 aa, Homo sapiens
  C08 VH region
EVQLLESGGGLVQPGRSLRLSCAASGFTVSSNYMSWVRQAPGKGLEWVSVIYSGGSTYYADSVKGRFTISRDNSKNTLYLQMNSLRAEDTAVYYCASPIELGAFDIWGQGTLVTVSS

SEQ ID NO: 64 - protein, 120 aa, Homo sapiens
  G04 VH region
QVQLQQSGPGLVKPSQTLSLTCAISGDSVSSKSAAWNWIRQSPSRGLEWLGRTYYRSKWSTDYAASVKSRITINPDTSKNQLSLQLNSVTPEDTAVYYCARTWSGYVDVWGQGTLVTVSS

SEQ ID NO: 65 - protein, 118 aa, Homo sapiens
  B07 VH region
EVQLLESGGGLVKPGGSLRLSCAASGFTFSDYYMSWIRQAPGKGLEWVSYISSSGSTIYYADSVKGRFTISRDNAKNSLYLQMNSLRAEDTAVYYCARENYLNAFDIWGRGTLVTVSS

SEQ ID NO: 66 - protein, 117 aa, Homo sapiens
  C05 VH region
EVQLLESGGGLVQPGGSLRLSCAASGFTFSSYAMSWVRQAPGKGLEWVSAISGGGGTTYSSDSVKGRFTISRDNSKNTLYLQMNSLRAEDTAVYYCARDSGVAFDIWGQGTLVTVSS

SEQ ID NO: 67 - protein, 119 aa, Homo sapiens
  E01 VH region
QVQLVQSGAEVKKPGESLKISCKGSGYSFTSYWIGWVRQMPGKGLEWMGIIYPGDSDTRYSPSFQGQVTISADKSISTAYLQWSSLKASDTAMYYCARHQVDTRTADYWGQGTLVTVSS

SEQ ID NO: 68 - protein, 120 aa, Homo sapiens
  E04 VH region
QVQLQQSGPGLVKPSQTLSLTCAISGDSVSSNSAAWNWIRQSPSRGLEWLGRTYYRSKWYNDYAVSVRSRITINPDTSKNQFSLQLNSVTPEDTAVYYCARSWNDAFDIWGQGTTVTVSS

SEQ ID NO: 69 - protein, 120 aa, Homo sapiens
  F07 VH region
QVQLQQSGPGLVKPSQTLSLTCVISGDSVSSNSAAWNWIRQSPSRGLEWLGRTYYRSKWYNDYAVSVKSRITINPDTSKNQFSLQLNSVTPEDTAVYYCARDYYYSMDVWGQGTMVTVSS

SEQ ID NO: 70 - protein, 118 aa, Homo sapiens
  G06 VH region
QVQLVESGGGLVKPGGSLRLSCAASGFTFSDYYMSWIRQAPGKGLEWVSYISSSGSTIYYADSVKGRFTISRDNAKNSLYLQMNSLRAEDTAVYYCARHSWNDAFDVWGQGTLVTVSS

SEQ ID NO: 71 - protein, 120 aa, Homo sapiens
  G09 VH region
QVQLQQSGPGLVKPSQTLSLTCAISGDSVSSNSAAWNWIRQSPSRGLEWLGRTYYGSKWYNEYALSVKSRIIINPDTSKNQFSLQLNSVTPEDTAVYYCARDYYYSMDVWGQGTLVTVSS

SEQ ID NO: 72 - protein, 118 aa, Homo sapiens
  B09 VH region
EVQLLESGGGLVKPGGSLRLSCAASGFTFSDYYMSWIRQAPGKGLEWVSYISSSGSTIYYADSVKGRFTISRDNAKNSLYLQMNSLRAEDTAVYYCARHSWSDAFDIWGQGTLVTVSS

SEQ ID NO: 73 - protein, 118 aa, Homo sapiens
  G10 VH region
EVQLVESGGGLVQPGGSLRLSCAASGFTFSDYYMSWIRQAPGKGLEWVSYISSSGSTIYYADSVKGRFTISRDNAKNSLYLQMNSLRAEDTAVYYCARHSWNDAFDIWGRGTLVTVSS

SEQ ID NO: 74 - protein, 109 aa, Homo sapiens
  E07 VL region
ASDIQMTQSPSSLSASVGDRVTIACRAGQSIGTYLNWYQQKPGKAPKLLIYVASSLQSGVPSRFSGSGSGTEFTLTISSLQPEDFATYYCQQSYSTLLTFGRGTKVEIK

SEQ ID NO: 75 - protein, 110 aa, Homo sapiens
  C08 VL region
ASSYELTQPPSVSVAPGKTARITCGGNNIGSQSVHWYQQKPGQAPMLVIYYDSDRPSGIPERFSGSNSGNTATLTISRVEAGDEADYYCQVWDSSSDHVVFGGGTKLTVL

SEQ ID NO: 76 - protein, 110 aa, Homo sapiens
  G04 VL region
ASDIQMTQSPPALSASVGDRVTITCRASQDINDWLAWYQHKPGKAPKLLIYDASSLESGVPSRFSGSGSGTEFTLTISSLQPDDFATYYCQQSYSTPQVTFGQGTRLEIK

SEQ ID NO: 77 - protein, 109 aa, Homo sapiens
  B07 VL region
ASDIQMTQSPSSLSASVGDRVTITCRTSQSLSNYLNWYQQKPGKAPKLLIYAASSLQSGVPSRFSGSGSGTDFTLTISSLQPEDFATYYCQQSYSTPLTFGGGTKLEIK

SEQ ID NO: 78 - protein, 109 aa, Homo sapiens
  C05 VL region
ASDIQMTQSPSFLSASVGDRVTITCRASQNIRTWLAWYQQKPGRAPKLLIYDASSLESGVPSRFSGSGSGTDFTLTISSLQPEDFATYYCQQFKRYPPTFGLGTKVEIK

SEQ ID NO: 79 - protein, 112 aa, Homo sapiens
  E01 VL region
ASQSALTQPASVSGSPGQSVTISCTGTRSDVGGYNYVSWYQHHPGKAPKLMIYEVSNRPSGVSNRFSGSKSGNTASLTISGLQAEDEADYYCSSYTSTSTLVFGGGTKLTVL

SEQ ID NO: 80 - protein, 109 aa, Homo sapiens
  E04 VL region
ASDIVMTQSPSTLSASIGDRVTITCRAGQSISTWLAWYQQKPGKAPKLLIYDASSLESGVPLRFSGSGSGTDFTLTISSLQPEDFATYYCQQSYSTPLTFGGGTKVEIK

SEQ ID NO: 81 - protein, 109 aa, Homo sapiens
  F07 VL region
ASDIQMTQSPSTLSASVGDRVTITCRASQSISSWLAWYQQKPGKAPKLLIYDASSLESGVPLRFSGSGSGTEFTLTISSLQPDDFATYYCQQSHSHPPTFGPGTKVDIK

SEQ ID NO: 82 - protein, 109 aa, Homo sapiens
  G06 VL region
ASDIQMTQSPSSLSASVGDRVSITCRASQSISSYLNWYQQKPGKAPKLLIYAASSLQSGVPSRFSGSGSGTDFTLTISSLQPEDFATYYCQQSYSTPDTFGGGTKVEIK

SEQ ID NO: 83 - protein, 109 aa, Homo sapiens
  G09 VL region
ASDIVMTQSPSTLSASIGDRVTITCRAGQSISTWLAWYQQKPGKAPKLLIYDASSLESGVPLRFSGSGSGTEFTLAISSLQPDDFATYYCQQSYSTPVTFGQGTKVEIK

SEQ ID NO: 84 - protein, 109 aa, Homo sapiens
  B09 VL region
ASDIQMTQSPSSLSASVGDRVTITCQASQDISNYLNWYQQKPGKAPKLLIYDASNLETGVPSRFSGSGSGTDFTLTISSLQPEDFATYYCQQSYSTPLTFGGGTKVEIK

SEQ ID NO: 85 - protein, 109 aa, Homo sapiens
  G10 VL region
ASDIQMTQSPSSLSASVGDRVTITCRASQSISSHLNWYQQKPGKAPKLLIYAASSLQSGVPSRFSASGSGTDFTLTISSLQPEDFATYYCQQSYSTLLTFGGGTKVEIK

SEQ ID NO: 86 - protein, 240 aa, Homo sapiens
  E07 scfv
QVQLVESGGGLVKPGGSLRLSCAASGFTFSDYYMSWIRQAPGKGLEWVSYISSSGSTIYYADSVKGRFTISRDNAKNSLYLQMNSLRAEDTAVYYCARVDYADAFDIWGQGTLVTVSSGGGGSGGGGSGGGASDIQMTQSPSSLSASVGDRVTIACRAGQSIGTYLNWYQQKPGKAPKLLIYVASSLQSGVPSRFSGSGSGTEFTLTISSLQPEDFATYYCQQSYSTLLTFGRGTKVEIK

SEQ ID NO: 87 - protein, 240 aa, Homo sapiens
  C08 scfv
EVQLLESGGGLVQPGRSLRLSCAASGFTVSSNYMSWVRQAPGKGLEWVSVIYSGGSTYYADSVKGRFTISRDNSKNTLYLQMNSLRAEDTAVYYCASPIELGAFDIWGQGTLVTVSSGGGGSGGGGSGGGASSYELTQPPSVSVAPGKTARITCGGNNIGSQSVHWYQQKPGQAPMLVIYYDSDRPSGIPERFSGSNSGNTATLTISRVEAGDEADYYCQVWDSSSDHVVFGGGTKLTVL

SEQ ID NO: 88 - protein, 243 aa, Homo sapiens
  G04 scfv
QVQLQQSGPGLVKPSQTLSLTCAISGDSVSSKSAAWNWIRQSPSRGLEWLGRTYYRSKWSTDYAASVKSRITINPDTSKNQLSLQLNSVTPEDTAVYYCARTWSGYVDVWGQGTLVTVSSGGGGSGGGGSGGGASDIQMTQSPPALSASVGDRVTITCRASQDINDWLAWYQHKPGKAPKLLIYDASSLESGVPSRFSGSGSGTEFTLTISSLQPDDFATYYCQQSYSTPQVTFGQGTRLEIK

SEQ ID NO: 89 - protein, 240 aa, Homo sapiens
  B07 scfv
EVQLLESGGGLVKPGGSLRLSCAASGFTFSDYYMSWIRQAPGKGLEWVSYISSSGSTIYYADSVKGRFTISRDNAKNSLYLQMNSLRAEDTAVYYCARENYLNAFDIWGRGTLVTVSSGGGGSGGGGSGGGASDIQMTQSPSSLSASVGDRVTITCRTSQSLSNYLNWYQQKPGKAPKLLIYAASSLQSGVPSRFSGSGSGTDFTLTISSLQPEDFATYYCQQSYSTPLTFGGGTKLEIK

SEQ ID NO: 90 - protein, 239 aa, Homo sapiens
  C05 scfv
EVQLLESGGGLVQPGGSLRLSCAASGFTFSSYAMSWVRQAPGKGLEWVSAISGGGGTTYSSDSVKGRFTISRDNSKNTLYLQMNSLRAEDTAVYYCARDSGVAFDIWGQGTLVTVSSGGGGSGGGGSGGGASDIQMTQSPSFLSASVGDRVTITCRASQNIRTWLAWYQQKPGRAPKLLIYDASSLESGVPSRFSGSGSGTDFTLTISSLQPEDFATYYCQQFKRYPPTFGLGTKVEIK

SEQ ID NO: 91 - protein, 244 aa, Homo sapiens
  E01 scfv
QVQLVQSGAEVKKPGESLKISCKGSGYSFTSYWIGWVRQMPGKGLEWMGIIYPGDSDTRYSPSFQGQVTISADKSISTAYLQWSSLKASDTAMYYCARHQVDTRTADYWGQGTLVTVSSGGGGSGGGGSGGGASQSALTQPASVSGSPGQSVTISCTGTRSDVGGYNYVSWYQHHPGKAPKLMIYEVSNRPSGVSNRFSGSKSGNTASLTISGLQAEDEADYYCSSYTSTSTLVFGGGTKLTVL

SEQ ID NO: 92 - protein, 242 aa, Homo sapiens
  E04 scfv
QVQLQQSGPGLVKPSQTLSLTCAISGDSVSSNSAAWNWIRQSPSRGLEWLGRTYYRSKWYNDYAVSVRSRITINPDTSKNQFSLQLNSVTPEDTAVYYCARSWNDAFDIWGQGTTVTVSSGGGGSGGGGSGGGASDIVMTQSPSTLSASIGDRVTITCRAGQSISTWLAWYQQKPGKAPKLLIYDASSLESGVPLRFSGSGSGTDFTLTISSLQPEDFATYYCQQSYSTPLTFGGGTKVEIK

SEQ ID NO: 93 - protein, 242 aa, Homo sapiens
  F07 scfv
QVQLQQSGPGLVKPSQTLSLTCVISGDSVSSNSAAWNWIRQSPSRGLEWLGRTYYRSKWYNDYAVSVKSRITINPDTSKNQFSLQLNSVTPEDTAVYYCARDYYYSMDVWGQGTMVTVSSGGGGSGGGGSGGGASDIQMTQSPSTLSASVGDRVTITCRASQSISSWLAWYQQKPGKAPKLLIYDASSLESGVPLRFSGSGSGTEFTLTISSLQPDDFATYYCQQSHSHPPTFGPGTKVDIK

SEQ ID NO: 94 - protein, 240 aa, Homo sapiens
  G06 scfv
QVQLVESGGGLVKPGGSLRLSCAASGFTFSDYYMSWIRQAPGKGLEWVSYISSSGSTIYYADSVKGRFTISRDNAKNSLYLQMNSLRAEDTAVYYCARHSWNDAFDVWGQGTLVTVSSGGGGSGGGGSGGGASDIQMTQSPSSLSASVGDRVSITCRASQSISSYLNWYQQKPGKAPKLLIYAASSLQSGVPSRFSGSGSGTDFTLTISSLQPEDFATYYCQQSYSTPDTFGGGTKVEIK

SEQ ID NO: 95 - protein, 242 aa, Homo sapiens
  G09 scfv
QVQLQQSGPGLVKPSQTLSLTCAISGDSVSSNSAAWNWIRQSPSRGLEWLGRTYYGSKWYNEYALSVKSRIIINPDTSKNQFSLQLNSVTPEDTAVYYCARDYYYSMDVWGQGTLVTVSSGGGGSGGGGSGGGASDIVMTQSPSTLSASIGDRVTITCRAGQSISTWLAWYQQKPGKAPKLLIYDASSLESGVPLRFSGSGSGTEFTLAISSLQPDDFATYYCQQSYSTPVTFGQGTKVEIK

SEQ ID NO: 96 - protein, 240 aa, Homo sapiens
  B09 scfv
EVQLLESGGGLVKPGGSLRLSCAASGFTFSDYYMSWIRQAPGKGLEWVSYISSSGSTIYYADSVKGRFTISRDNAKNSLYLQMNSLRAEDTAVYYCARHSWSDAFDIWGQGTLVTVSSGGGGSGGGGSGGGASDIQMTQSPSSLSASVGDRVTITCQASQDISNYLNWYQQKPGKAPKLLIYDASNLETGVPSRFSGSGSGTDFTLTISSLQPEDFATYYCQQSYSTPLTFGGGTKVEIK

SEQ ID NO: 97 - protein, 240 aa, Homo sapiens
  G10 scfv
EVQLVESGGGLVQPGGSLRLSCAASGFTFSDYYMSWIRQAPGKGLEWVSYISSSGSTIYYADSVKGRFTISRDNAKNSLYLQMNSLRAEDTAVYYCARHSWNDAFDIWGRGTLVTVSSGGGGSGGGGSGGGASDIQMTQSPSSLSASVGDRVTITCRASQSISSHLNWYQQKPGKAPKLLIYAASSLQSGVPSRFSASGSGTDFTLTISSLQPEDFATYYCQQSYSTLLTFGGGTKVEIK

SEQ ID NO: 98 - protein, 13 aa, Artificial Sequence
  Synthetic linker
GGGGSGGGGSGGG

SEQ ID NO: 99 - DNA, 765 bp, Homo sapiens
  E07 nucleotide
gccatggcccaggtgcagctggtggagtctgggggaggcttggtcaagcctggagggtccctgagactctcctgtgcagcctctggattcaccttcagtgactactacatgagctggatccgccaggctccagggaaggggctggagtgggtttcatacattagtagtagtggtagtaccatatactacgcagactctgtgaagggccgattcaccatctccagggacaacgccaagaactcactgtatctgcaaatgaacagcctgagagccgaggacacggctgtgtattactgtgcaagggtggactacgctgatgcatttgatatctggggccagggcaccctggtcaccgtctcgagtggtggaggcggttcaggcggaggtggctctggcggtggcgctagcgacatccagatgacccagtctccatcctccctgtctgcatctgtaggagacagagtcaccatcgcttgccgggcaggtcagagcattggcacctatttaaattggtatcagcagaaaccagggaaagcccctaaactcctgatctatgttgcatccagtttgcaaagtggggtcccgtcacggttcagtggcagtggatctgggacagaattcactctcaccatcagcagtctgcaacctgaagattttgcaacttactactgtcaacagagttacagtaccctcctcactttcggcagagggaccaaggtggaaatcaaacgtaccgcggccgcatccgcacatcatcatcaccat

SEQ ID NO: 100 - DNA, 768 bp, Homo sapiens
  C08 nucleotide
gccatggccgaggtgcagctgttggagtctgggggaggcttggtacagcctggcaggtccctgagactctcctgtgcagcctctgggttcaccgtcagtagcaactacatgagctgggtccgccaggctccagggaaggggctggagtgggtctcagttatttatagcggtggtagcacatactacgcagactccgtgaagggccgattcaccatctccagagacaattccaagaacacgctgtatcttcaaatgaacagcctgagagccgaggacacggctgtgtattactgtgcgagccccatagagctgggtgcttttgatatctggggccaaggaaccctggtcaccgtctcgagtggtggaggcggttcaggcggaggtggctctggcggtggcgctagctcctatgagctgactcagccaccctcagtgtcagtggccccaggaaagacggccaggattacctgtgggggaaacaacattggaagtcaaagtgtgcactggtaccagcagaagccaggccaggcccctatgctggtcatctattatgatagcgaccggccctcagggatccctgagcgattctctggctccaactctgggaacacggccaccctgaccatcagcagggtcgaagccggggatgaggccgactattactgtcaggtgtgggatagtagtagtgatcatgtggtattcggcggcgggaccaagctgaccgtcctaggtcagcccgcggccgcatccgcacatcatcatcaccat

SEQ ID NO: 101 - DNA, 774 bp, Homo sapiens
  G04 nucleotide
gccatggcccaggtacagctgcagcagtcaggtccaggactggtgaagccctcgcagaccctctcactcacctgtgccatctccggggacagtgtctccagcaaaagtgctgcttggaactggatcaggcagtccccatcgagaggccttgagtggctgggaaggacatactacaggtccaagtggtctactgattatgcagcatctgtgaaaagtcgaataaccatcaacccagacacatccaagaaccagctctccctgcagttaaactctgtgactcccgaggacacggctgtgtattactgtgcaagaacgtggagtggttatgtggacgtctggggccaaggaaccctggtcaccgtctcgagtggtggaggcggttcaggcggaggtggctctggcggtggcgctagcgacatccagatgacccagtcccctcccgccctgtctgcatctgtgggagacagagtcaccatcacttgccgggccagtcaagatattaatgactggttggcctggtatcagcataaacctgggaaagcccctaagctcctgatctatgatgcctccagtttggaaagtggggtcccatcaaggttcagcggcagtggatctgggacagaattcactctcaccatcagcagcctgcagcctgatgattttgcaacttactactgtcaacagagttacagtacccctcaggtcacttttggccaggggacacgactggagatcaaacgtaccgcggccgcatccgcacatcatcatcaccat

SEQ ID NO: 102 - DNA, 765 bp, Homo sapiens
  B07 nucleotide
gccatggccgaggtgcagctgttggagtctgggggaggcttggtcaagcctggagggtccctgagactctcctgtgcggcctctggattcaccttcagtgactactacatgagctggatccgccaggctccagggaaggggctggagtgggtttcatacattagtagtagtggtagtaccatatactacgcagactctgtgaagggccgattcaccatctccagggacaacgccaagaactcactgtatctgcaaatgaacagcctgagagccgaggacacggccgtgtattactgtgcgagagaaaactatctaaatgcttttgatatctggggccgtggcaccctggtcaccgtctcgagtggtggaggcggttcaggcggaggtggctctggcggtggcgctagcgacatccagatgacccagtctccatcctccctgtctgcatctgtaggagacagagtcaccatcacttgccggacaagtcagagccttagtaattacttaaattggtatcagcagaaaccagggaaagcccctaagctcctgatctatgctgcatccagtttgcaaagtggggtcccatcaaggttcagtggcagtggatctgggacagatttcactctcaccatcagcagtctgcaacctgaagattttgcgacttactactgtcaacagagttacagtacccctctcactttcggcggagggaccaagctagagatcaaacgtaccgcggccgcatccgcacatcatcatcaccat

SEQ ID NO: 103 - DNA, 762 bp, Homo sapiens
  C05 nucleotide
gccatggccgaggtgcagctgttggagtctgggggaggcttggtacagcctggggggtccctgagactctcctgtgcagcctctggattcacctttagcagctatgccatgagctgggtccgccaggctccagggaaggggctggagtgggtctcagctattagtggtggtggtggtaccacatactcctcagactccgtgaagggccggttcaccatctccagagacaattccaagaacacgctgtatctgcaaatgaacagcctgagagccgaggacacggctgtgtattactgtgcgagagattcaggggttgcttttgatatctggggccaaggaaccctggtcaccgtctcgagtggtggaggcggttcaggcggaggtggctctggcggtggcgctagcgacatccagatgacccagtctccatccttcctgtctgcatctgtaggagacagagtcaccatcacttgccgggccagtcagaatatacgtacctggttggcctggtatcagcagaaaccagggagagcccctaagctcctgatctatgatgcctccagtttggaaagtggggtcccatcaaggttcagcggcagtggatctgggactgatttcactctcaccatcagcagcctgcagcctgaagattttgcaacttattactgtcaacagtttaaacgttaccctccgacgtttggcctggggaccaaggtggagatcaaacgtaccgcggccgcatccgcacatcatcatcaccat

SEQ ID NO: 104 - DNA, 780 bp, Homo sapiens
  E01 nucleotide
gccatggcccaggtccagctggtacagtctggagcagaggtgaaaaagcccggggagtctctgaagatctcctgtaagggttctggatacagctttaccagctactggatcggctgggtgcgccagatgcccgggaaaggcctggagtggatggggatcatctatcctggtgactctgataccagatacagcccgtccttccaaggccaggtcaccatctcagccgacaagtccatcagcaccgcctacctgcagtggagcagcctgaaggcctcggacaccgccatgtattattgtgcgagacatcaggttgatacacggacggctgattactggggccagggaaccctggtcaccgtctcgagtggtggaggcggttcaggcggaggtggctctggcggtggcgctagccagtctgcgctgactcagcctgcctccgtgtctgggtctcctggacagtcggtcaccatctcctgcactggaaccaggagtgacgttggtggttataactatgtctcctggtaccaacaccacccaggcaaagcccccaaactcatgatttatgaggtcagtaatcggccctcaggggtttctaatcgcttctctggctccaagtctggcaacacggcctccctgaccatctctgggctccaggctgaggacgaggctgattattactgcagctcatatacaagcaccagcactctggtattcggcggagggaccaagctgaccgtcctaggtcagcccgcggccgcatccgcacatcatcatcaccat

SEQ ID NO: 105 - DNA, 771 bp, Homo sapiens
  E04 nucleotide
gccatggcccaggtacagctgcagcagtcaggtccaggactggtgaagccctcgcagaccctctcactcacctgtgccatctccggggacagtgtctctagcaacagtgctgcttggaactggatcaggcagtccccatcgagaggccttgagtggctgggaaggacatactacaggtccaagtggtataatgattatgcagtatctgtgagaagtcgaataaccatcaacccagacacatccaagaaccagttctccctgcagctgaactctgtgactcccgaggacacggctgtgtattactgtgcaagaagctggaatgatgcttttgatatctgggggcaagggaccacggtcaccgtctcgagtggtggaggcggttcaggcggaggtggctctggcggtggcgctagcgatattgtgatgacacagtctccttccaccctgtctgcatctataggagacagagtcaccatcacttgccgggccggtcagagtattagtacctggttggcctggtatcagcagaaaccagggaaagcccctaagctcctgatctatgatgcctccagtttggaaagtggggtcccattaaggttcagcggcagtggatctgggacagatttcactctcaccatcagcagtctgcaacctgaagattttgcaacttactactgtcaacagagttacagtaccccgctcactttcggcggagggaccaaggtggagatcaaacgtaccgcggccgcatccgcacatcatcatcaccat

SEQ ID NO: 106 - DNA, 771 bp, Homo sapiens
  F07 nucleotide
gccatggcccaggtacagctgcagcagtcaggtccaggcctggtgaagccctcgcagaccctctcactcacctgtgtcatctccggggacagtgtctctagcaacagtgctgcttggaactggatcaggcagtccccatcgcgaggccttgagtggctgggaaggacatactacaggtccaagtggtataatgattatgcagtatctgtgaaaagtcgaataaccatcaacccagacacatccaagaaccagttctccctgcagctgaactctgtgactcccgaggacacggctgtctattattgtgcaagagactactactacagtatggacgtctggggccaagggacaatggtcaccgtctcgagtggtggaggcggttcaggcggaggtggctctggcggtggcgctagcgacatccagatgacccagtctccctccaccctgtctgcatctgtaggagacagagtcaccatcacttgccgggccagtcagagtattagtagctggttggcctggtatcagcagaaaccagggaaagcccctaagctcctgatctatgatgcctccagtttggaaagtggggtcccattaaggttcagcggcagtggatctgggacagaattcactctcaccatcagcagcctgcagcctgatgattttgcaacttattactgtcaacagagtcacagtcacccccctactttcggccctgggaccaaagtggatatcaaacgtaccgcggccgcatccgcacatcatcatcaccat

SEQ ID NO: 107 - DNA, 765 bp, Homo sapiens
  G06 nucleotide
gccatggcccaggtgcagctggtggagtctgggggaggcttggtcaagcctggagggtccctgagactctcctgtgcagcctctggattcaccttcagtgactactacatgagctggatccgccaggctccagggaaggggctggagtgggtttcatacattagtagtagtggtagtaccatatactacgcagactctgtgaagggccgattcaccatctccagggacaacgccaagaactcactgtatctgcaaatgaacagcctgagagccgaggacacggccgtgtattactgtgcgagacatagctggaatgatgcttttgatgtctggggccagggaaccctggtcaccgtctcgagtggtggaggcggttcaggcggaggtggctctggcggtggcgctagcgacatccagatgacccagtctccatcctccctgtctgcatctgtaggagacagagtctccatcacctgccgggcaagtcagagcattagcagctatttaaattggtatcagcagaaaccagggaaagcccctaagctcctgatctatgctgcatccagtttgcaaagtggggtcccatcaaggttcagtggcagtggatctgggacagatttcactctcaccatcagcagtctgcaacctgaagattttgcaacttactactgtcagcagagttacagtacccccgacactttcggcggagggaccaaggtggaaatcaaacgtaccgcggccgcatccgcacatcatcatcaccat

SEQ ID NO: 108 - DNA, 771 bp, Homo sapiens
  G09 nucleotide
gccatggcccaggtacagctgcagcagtcaggtccaggactggtgaagccctcgcagaccctctcactcacctgtgccatctccggggacagtgtctctagcaacagtgctgcttggaactggatcaggcagtccccatcgagaggccttgagtggctgggaaggacatactacgggtccaagtggtataatgagtatgcactatctgtgaaaagtcgaataatcatcaacccagacacatccaagaaccagttctccctgcagctgaactctgtgactcccgaggacacggctgtctattattgtgcaagagactactactacagtatggacgtctggggccagggaaccctggtcaccgtctcgagtggtggaggcggttcaggcggaggtggctctggcggtggcgctagcgatattgtgatgactcagtctccttccaccctgtctgcatctataggagacagagtcaccatcacttgccgggccggtcagagtattagtacctggttggcctggtatcagcagaaaccagggaaagcccctaagctcctgatctatgatgcctccagtttggaaagtggggtcccattaaggttcagcggcagtggatctgggacagaattcactctcgccatcagcagcctgcagcctgatgattttgcaacttactactgtcaacagagttacagtaccccggtaacttttggccaggggaccaaggtggagatcaaacgtaccgcggccgcatccgcacatcatcatcaccat

SEQ ID NO: 109 - DNA, 765 bp, Homo sapiens
  B09 nucleotide
gccatggccgaggtgcagctgttggagtctgggggaggcttggtcaagcctggagggtccctgagactctcctgtgcagcctctggattcaccttcagtgactactacatgagctggatccgccaggctccagggaaggggctggagtgggtttcatacattagtagtagtggtagtaccatatactacgcagactctgtgaagggccgattcaccatctccagggacaacgccaagaactcactgtatctgcaaatgaacagcctgagagccgaggacacggccgtgtattactgtgcgagacatagctggagtgatgcttttgatatctggggccaaggaaccctggtcaccgtctcgagtggtggaggcggttcaggcggaggtggctctggcggtggcgctagcgacatccagatgacccagtctccatcctccctgtctgcatctgtaggagacagagtcaccatcacttgccaggcgagtcaggacattagcaactatttaaattggtatcagcagaaaccagggaaagcccctaagctcctgatctacgatgcatccaatttggaaacaggggtcccatcaaggttcagtggaagtggatctgggacagatttcactctcaccatcagcagtctgcaacctgaagattttgcaacttactactgtcaacagagttacagtactcctctcactttcggcggagggaccaaggtggagatcaaacgtaccgcggccgcatccgcacatcatcatcaccat

SEQ ID NO: 110 - DNA, 765 bp, Homo sapiens
  G10 nucleotide
gccatggccgaagtgcagctggtggagtccgggggaggcttagttcagcctggggggtccctgagactctcctgtgcagcctctggattcaccttcagtgactactacatgagctggatccgccaggctccagggaaggggctggagtgggtttcatacattagtagtagtggtagtaccatatactacgcagactctgtgaagggccgattcaccatctccagggacaacgccaagaactcactgtatctgcaaatgaacagcctgagagccgaggacacggccgtgtattactgtgcgagacatagctggaatgatgcttttgatatctggggccgtggcaccctggtcaccgtctcgagtggtggaggcggttcaggcggaggtggctctggcggtggcgctagcgacatccagatgacccagtctccatcctccctgtctgcatctgtaggagacagagtcaccatcacttgccgggcaagtcagagcattagcagccatttaaattggtatcagcagaaaccagggaaagcccctaagctcctgatctatgctgcatccagtttgcaaagtggggtcccatccaggttcagtgccagtggatctgggacagatttcactctcaccatcagcagcctgcagcctgaagattttgcaacttactactgtcaacagagttacagtaccctgctcactttcggcggagggaccaaggtggaaatcaaacgtaccgcggccgcatccgcacatcatcatcaccat

SEQ ID NO: 111 - protein, 664 aa, Homo sapiens
  E07 full heavy and light
ASDIQMTQSPSSLSASVGDRVTIACRAGQSIGTYLNWYQQKPGKAPKLLIYVASSLQSGVPSRFSGSGSGTEFTLTISSLQPEDFATYYCQQSYSTLLTFGRGTKVEIKRTAAAPSVFIFPPSDEQLKSGTASVVCLLNNFYPREAKVQWKVDNALQSGNSQESVTEQDSKDSTYSLSSTLTLSKADYEKHKLYACEVTHQGLSSPVTKSFNRGECQVQLVESGGGLVKPGGSLRLSCAASGFTFSDYYMSWIRQAPGKGLEWVSYISSSGSTIYYADSVKGRFTISRDNAKNSLYLQMNSLRAEDTAVYYCARVDYADAFDIWGQGTLVTVSSASTKGPSVFPLAPSSKSTSGGTAALGCLVKDYFPEPVTVSWNSGALTSGVHTFPAVLQSSGLYSLSSVVTVPSSSLGTQTYICNVNHKPSNTKVDKKVEPKSCDKTHTCPPCPAPELLGGPSVFLFPPKPKDTLMISRTPEVTCVVVDVSHEDPEVKFNWYVDGVEVHNAKTKPREEQYNSTYRVVSVLTVLHQDWLNGKEYKCKVSNKALPAPIEKTISKAKGQPREPQVYTLPPSRDELTKNQVSLTCLVKGFYPSDIAVEWESNGQPENNYKTTPPVLDSDGSFFLYSKLTVDKSRWQQGNVFSCSVMHEALHNHYTQKSLSLSPGK

SEQ ID NO: 112 - protein, 667 aa, Homo sapiens
  C08 full heavy and light
ASDIQMTQSPPALSASVGDRVTITCRASQDINDWLAWYQHKPGKAPKLLIYDASSLESGVPSRFSGSGSGTEFTLTISSLQPDDFATYYCQQSYSTPQVTFGQGTRLEIKRTAAAPSVFIFPPSDEQLKSGTASVVCLLNNFYPREAKVQWKVDNALQSGNSQESVTEQDSKDSTYSLSSTLTLSKADYEKHKLYACEVTHQGLSSPVTKSFNRGECQVQLQQSGPGLVKPSQTLSLTCAISGDSVSSKSAAWNWIRQSPSRGLEWLGRTYYRSKWSTDYAASVKSRITINPDTSKNQLSLQLNSVTPEDTAVYYCARTWSGYVDVWGQGTLVTVSSASTKGPSVFPLAPSSKSTSGGTAALGCLVKDYFPEPVTVSWNSGALTSGVHTFPAVLQSSGLYSLSSVVTVPSSSLGTQTYICNVNHKPSNTKVDKKVEPKSCDKTHTCPPCPAPELLGGPSVFLFPPKPKDTLMISRTPEVTCVVVDVSHEDPEVKFNWYVDGVEVHNAKTKPREEQYNSTYRVVSVLTVLHQDWLNGKEYKCKVSNKALPAPIEKTISKAKGQPREPQVYTLPPSRDELTKNQVSLTCLVKGFYPSDIAVEWESNGQPENNYKTTPPVLDSDGSFFLYSKLTVDKSRWQQGNVFSCSVMHEALHNHYTQKSLSLSPGK

SEQ ID NO: 113 - protein, 664 aa, Homo sapiens
  G04 full heavy and light
ASDIQMTQSPSSLSASVGDRVTITCRTSQSLSNYLNWYQQKPGKAPKLLIYAASSLQSGVPSRFSGSGSGTDFTLTISSLQPEDFATYYCQQSYSTPLTFGGGTKLEIKRTAAAPSVFIFPPSDEQLKSGTASVVCLLNNFYPREAKVQWKVDNALQSGNSQESVTEQDSKDSTYSLSSTLTLSKADYEKHKLYACEVTHQGLSSPVTKSFNRGECEVQLLESGGGLVKPGGSLRLSCAASGFTFSDYYMSWIRQAPGKGLEWVSYISSSGSTIYYADSVKGRFTISRDNAKNSLYLQMNSLRAEDTAVYYCARENYLNAFDIWGRGTLVTVSSASTKGPSVFPLAPSSKSTSGGTAALGCLVKDYFPEPVTVSWNSGALTSGVHTFPAVLQSSGLYSLSSVVTVPSSSLGTQTYICNVNHKPSNTKVDKKVEPKSCDKTHTCPPCPAPELLGGPSVFLFPPKPKDTLMISRTPEVTCVVVDVSHEDPEVKFNWYVDGVEVHNAKTKPREEQYNSTYRVVSVLTVLHQDWLNGKEYKCKVSNKALPAPIEKTISKAKGQPREPQVYTLPPSRDELTKNQVSLTCLVKGFYPSDIAVEWESNGQPENNYKTTPPVLDSDGSFFLYSKLTVDKSRWQQGNVFSCSVMHEALHNHYTQKSLSLSPGK

SEQ ID NO: 114 - protein, 663 aa, Homo sapiens
  B07 full heavy and light
ASDIQMTQSPSFLSASVGDRVTITCRASQNIRTWLAWYQQKPGRAPKLLIYDASSLESGVPSRFSGSGSGTDFTLTISSLQPEDFATYYCQQFKRYPPTFGLGTKVEIKRTAAAPSVFIFPPSDEQLKSGTASVVCLLNNFYPREAKVQWKVDNALQSGNSQESVTEQDSKDSTYSLSSTLTLSKADYEKHKLYACEVTHQGLSSPVTKSFNRGECEVQLLESGGGLVQPGGSLRLSCAASGFTFSSYAMSWVRQAPGKGLEWVSAISGGGGTTYSSDSVKGRFTISRDNSKNTLYLQMNSLRAEDTAVYYCARDSGVAFDIWGQGTLVTVSSASTKGPSVFPLAPSSKSTSGGTAALGCLVKDYFPEPVTVSWNSGALTSGVHTFPAVLQSSGLYSLSSVVTVPSSSLGTQTYICNVNHKPSNTKVDKKVEPKSCDKTHTCPPCPAPELLGGPSVFLFPPKPKDTLMISRTPEVTCVVVDVSHEDPEVKFNWYVDGVEVHNAKTKPREEQYNSTYRVVSVLTVLHQDWLNGKEYKCKVSNKALPAPIEKTISKAKGQPREPQVYTLPPSRDELTKNQVSLTCLVKGFYPSDIAVEWESNGQPENNYKTTPPVLDSDGSFFLYSKLTVDKSRWQQGNVFSCSVMHEALHNHYTQKSLSLSPGK

SEQ ID NO: 115 - protein, 667 aa, Homo sapiens
  C05 full heavy and light
ASQSALTQPASVSGSPGQSVTISCTGTRSDVGGYNYVSWYQHHPGKAPKLMIYEVSNRPSGVSNRFSGSKSGNTASLTISGLQAEDEADYYCSSYTSTSTLVFGGGTKLTVLGQPAAAPSVTLFPPSSEELQANKATLVCLISDFYPGAVTVAWKADSSPVKAGVETTTPSKQSNNKYAASSYLSLTPEQWKSHRSYSCQVTHEGSTVEKTVAPTECSQVQLVQSGAEVKKPGESLKISCKGSGYSFTSYWIGWVRQMPGKGLEWMGIIYPGDSDTRYSPSFQGQVTISADKSISTAYLQWSSLKASDTAMYYCARHQVDTRTADYWGQGTLVTVSSASTKGPSVFPLAPSSKSTSGGTAALGCLVKDYFPEPVTVSWNSGALTSGVHTFPAVLQSSGLYSLSSVVTVPSSSLGTQTYICNVNHKPSNTKVDKKVEPKSCDKTHTCPPCPAPELLGGPSVFLFPPKPKDTLMISRTPEVTCVVVDVSHEDPEVKFNWYVDGVEVHNAKTKPREEQYNSTYRVVSVLTVLHQDWLNGKEYKCKVSNKALPAPIEKTISKAKGQPREPQVYTLPPSRDELTKNQVSLTCLVKGFYPSDIAVEWESNGQPENNYKTTPPVLDSDGSFFLYSKLTVDKSRWQQGNVFSCSVMHEALHNHYTQKSLSLSPGK

SEQ ID NO: 116 - protein, 663 aa, Homo sapiens
  E01 full heavy and light
ASSYELTQPPSVSVAPGKTARITCGGNNIGSQSVHWYQQKPGQAPMLVIYYDSDRPSGIPERFSGSNSGNTATLTISRVEAGDEADYYCQVWDSSSDHVVFGGGTKLTVLGQPAAAPSVTLFPPSSEELQANKATLVCLISDFYPGAVTVAWKADSSPVKAGVETTTPSKQSNNKYAASSYLSLTPEQWKSHRSYSCQVTHEGSTVEKTVAPTECSEVQLLESGGGLVQPGRSLRLSCAASGFTVSSNYMSWVRQAPGKGLEWVSVIYSGGSTYYADSVKGRFTISRDNSKNTLYLQMNSLRAEDTAVYYCASPIELGAFDIWGQGTLVTVSSASTKGPSVFPLAPSSKSTSGGTAALGCLVKDYFPEPVTVSWNSGALTSGVHTFPAVLQSSGLYSLSSVVTVPSSSLGTQTYICNVNHKPSNTKVDKKVEPKSCDKTHTCPPCPAPELLGGPSVFLFPPKPKDTLMISRTPEVTCVVVDVSHEDPEVKFNWYVDGVEVHNAKTKPREEQYNSTYRVVSVLTVLHQDWLNGKEYKCKVSNKALPAPIEKTISKAKGQPREPQVYTLPPSRDELTKNQVSLTCLVKGFYPSDIAVEWESNGQPENNYKTTPPVLDSDGSFFLYSKLTVDKSRWQQGNVFSCSVMHEALHNHYTQKSLSLSPGK

SEQ ID NO: 117 - protein, 666 aa, Homo sapiens
  E04 full heavy and light
ASDIVMTQSPSTLSASIGDRVTITCRAGQSISTWLAWYQQKPGKAPKLLIYDASSLESGVPLRFSGSGSGTDFTLTISSLQPEDFATYYCQQSYSTPLTFGGGTKVEIKRTAAAPSVFIFPPSDEQLKSGTASVVCLLNNFYPREAKVQWKVDNALQSGNSQESVTEQDSKDSTYSLSSTLTLSKADYEKHKLYACEVTHQGLSSPVTKSFNRGECQVQLQQSGPGLVKPSQTLSLTCAISGDSVSSNSAAWNWIRQSPSRGLEWLGRTYYRSKWYNDYAVSVRSRITINPDTSKNQFSLQLNSVTPEDTAVYYCARSWNDAFDIWGQGTTVTVSSASTKGPSVFPLAPSSKSTSGGTAALGCLVKDYFPEPVTVSWNSGALTSGVHTFPAVLQSSGLYSLSSVVTVPSSSLGTQTYICNVNHKPSNTKVDKKVEPKSCDKTHTCPPCPAPELLGGPSVFLFPPKPKDTLMISRTPEVTCVVVDVSHEDPEVKFNWYVDGVEVHNAKTKPREEQYNSTYRVVSVLTVLHQDWLNGKEYKCKVSNKALPAPIEKTISKAKGQPREPQVYTLPPSRDELTKNQVSLTCLVKGFYPSDIAVEWESNGQPENNYKTTPPVLDSDGSFFLYSKLTVDKSRWQQGNVFSCSVMHEALHNHYTQKSLSLSPGK

SEQ ID NO: 118 - protein, 666 aa, Homo sapiens
  F07 full heavy and light
ASDIQMTQSPSTLSASVGDRVTITCRASQSISSWLAWYQQKPGKAPKLLIYDASSLESGVPLRFSGSGSGTEFTLTISSLQPDDFATYYCQQSHSHPPTFGPGTKVDIKRTAAAPSVFIFPPSDEQLKSGTASVVCLLNNFYPREAKVQWKVDNALQSGNSQESVTEQDSKDSTYSLSSTLTLSKADYEKHKLYACEVTHQGLSSPVTKSFNRGECQVQLQQSGPGLVKPSQTLSLTCVISGDSVSSNSAAWNWIRQSPSRGLEWLGRTYYRSKWYNDYAVSVKSRITINPDTSKNQFSLQLNSVTPEDTAVYYCARDYYYSMDVWGQGTMVTVSSASTKGPSVFPLAPSSKSTSGGTAALGCLVKDYFPEPVTVSWNSGALTSGVHTFPAVLQSSGLYSLSSVVTVPSSSLGTQTYICNVNHKPSNTKVDKKVEPKSCDKTHTCPPCPAPELLGGPSVFLFPPKPKDTLMISRTPEVTCVVVDVSHEDPEVKFNWYVDGVEVHNAKTKPREEQYNSTYRVVSVLTVLHQDWLNGKEYKCKVSNKALPAPIEKTISKAKGQPREPQVYTLPPSRDELTKNQVSLTCLVKGFYPSDIAVEWESNGQPENNYKTTPPVLDSDGSFFLYSKLTVDKSRWQQGNVFSCSVMHEALHNHYTQKSLSLSPGK

SEQ ID NO: 119 - protein, 664 aa, Homo sapiens
  G06 full heavy and light
ASDIQMTQSPSSLSASVGDRVSITCRASQSISSYLNWYQQKPGKAPKLLIYAASSLQSGVPSRFSGSGSGTDFTLTISSLQPEDFATYYCQQSYSTPDTFGGGTKVEIKRTAAAPSVFIFPPSDEQLKSGTASVVCLLNNFYPREAKVQWKVDNALQSGNSQESVTEQDSKDSTYSLSSTLTLSKADYEKHKLYACEVTHQGLSSPVTKSFNRGECQVQLVESGGGLVKPGGSLRLSCAASGFTFSDYYMSWIRQAPGKGLEWVSYISSSGSTIYYADSVKGRFTISRDNAKNSLYLQMNSLRAEDTAVYYCARHSWNDAFDVWGQGTLVTVSSASTKGPSVFPLAPSSKSTSGGTAALGCLVKDYFPEPVTVSWNSGALTSGVHTFPAVLQSSGLYSLSSVVTVPSSSLGTQTYICNVNHKPSNTKVDKKVEPKSCDKTHTCPPCPAPELLGGPSVFLFPPKPKDTLMISRTPEVTCVVVDVSHEDPEVKFNWYVDGVEVHNAKTKPREEQYNSTYRVVSVLTVLHQDWLNGKEYKCKVSNKALPAPIEKTISKAKGQPREPQVYTLPPSRDELTKNQVSLTCLVKGFYPSDIAVEWESNGQPENNYKTTPPVLDSDGSFFLYSKLTVDKSRWQQGNVFSCSVMHEALHNHYTQKSLSLSPGK

SEQ ID NO: 120 - protein, 666 aa, Homo sapiens
  G09 full heavy and light
ASDIVMTQSPSTLSASIGDRVTITCRAGQSISTWLAWYQQKPGKAPKLLIYDASSLESGVPLRFSGSGSGTEFTLAISSLQPDDFATYYCQQSYSTPVTFGQGTKVEIKRTAAAPSVFIFPPSDEQLKSGTASVVCLLNNFYPREAKVQWKVDNALQSGNSQESVTEQDSKDSTYSLSSTLTLSKADYEKHKLYACEVTHQGLSSPVTKSFNRGECQVQLQQSGPGLVKPSQTLSLTCAISGDSVSSNSAAWNWIRQSPSRGLEWLGRTYYGSKWYNEYALSVKSRIIINPDTSKNQFSLQLNSVTPEDTAVYYCARDYYYSMDVWGQGTLVTVSSASTKGPSVFPLAPSSKSTSGGTAALGCLVKDYFPEPVTVSWNSGALTSGVHTFPAVLQSSGLYSLSSVVTVPSSSLGTQTYICNVNHKPSNTKVDKKVEPKSCDKTHTCPPCPAPELLGGPSVFLFPPKPKDTLMISRTPEVTCVVVDVSHEDPEVKFNWYVDGVEVHNAKTKPREEQYNSTYRVVSVLTVLHQDWLNGKEYKCKVSNKALPAPIEKTISKAKGQPREPQVYTLPPSRDELTKNQVSLTCLVKGFYPSDIAVEWESNGQPENNYKTTPPVLDSDGSFFLYSKLTVDKSRWQQGNVFSCSVMHEALHNHYTQKSLSLSPGK

SEQ ID NO: 121 - protein, 664 aa, Homo sapiens
  B09 full heavy and light
ASDIQMTQSPSSLSASVGDRVTITCQASQDISNYLNWYQQKPGKAPKLLIYDASNLETGVPSRFSGSGSGTDFTLTISSLQPEDFATYYCQQSYSTPLTFGGGTKVEIKRTAAAPSVFIFPPSDEQLKSGTASVVCLLNNFYPREAKVQWKVDNALQSGNSQESVTEQDSKDSTYSLSSTLTLSKADYEKHKLYACEVTHQGLSSPVTKSFNRGECEVQLLESGGGLVKPGGSLRLSCAASGFTFSDYYMSWIRQAPGKGLEWVSYISSSGSTIYYADSVKGRFTISRDNAKNSLYLQMNSLRAEDTAVYYCARHSWSDAFDIWGQGTLVTVSSASTKGPSVFPLAPSSKSTSGGTAALGCLVKDYFPEPVTVSWNSGALTSGVHTFPAVLQSSGLYSLSSVVTVPSSSLGTQTYICNVNHKPSNTKVDKKVEPKSCDKTHTCPPCPAPELLGGPSVFLFPPKPKDTLMISRTPEVTCVVVDVSHEDPEVKFNWYVDGVEVHNAKTKPREEQYNSTYRVVSVLTVLHQDWLNGKEYKCKVSNKALPAPIEKTISKAKGQPREPQVYTLPPSRDELTKNQVSLTCLVKGFYPSDIAVEWESNGQPENNYKTTPPVLDSDGSFFLYSKLTVDKSRWQQGNVFSCSVMHEALHNHYTQKSLSLSPGK

SEQ ID NO: 122 - protein, 664 aa, Homo sapiens
  G10 full heavy and light
ASDIQMTQSPSSLSASVGDRVTITCRASQSISSHLNWYQQKPGKAPKLLIYAASSLQSGVPSRFSASGSGTDFTLTISSLQPEDFATYYCQQSYSTLLTFGGGTKVEIKRTAAAPSVFIFPPSDEQLKSGTASVVCLLNNFYPREAKVQWKVDNALQSGNSQESVTEQDSKDSTYSLSSTLTLSKADYEKHKLYACEVTHQGLSSPVTKSFNRGECEVQLVESGGGLVQPGGSLRLSCAASGFTFSDYYMSWIRQAPGKGLEWVSYISSSGSTIYYADSVKGRFTISRDNAKNSLYLQMNSLRAEDTAVYYCARHSWNDAFDIWGRGTLVTVSSASTKGPSVFPLAPSSKSTSGGTAALGCLVKDYFPEPVTVSWNSGALTSGVHTFPAVLQSSGLYSLSSVVTVPSSSLGTQTYICNVNHKPSNTKVDKKVEPKSCDKTHTCPPCPAPELLGGPSVFLFPPKPKDTLMISRTPEVTCVVVDVSHEDPEVKFNWYVDGVEVHNAKTKPREEQYNSTYRVVSVLTVLHQDWLNGKEYKCKVSNKALPAPIEKTISKAKGQPREPQVYTLPPSRDELTKNQVSLTCLVKGFYPSDIAVEWESNGQPENNYKTTPPVLDSDGSFFLYSKLTVDKSRWQQGNVFSCSVMHEALHNHYTQKSLSLSPGK

SEQ ID NO: 123 - protein, 254 aa, Artificial Sequence
  TRDV1(3OMZ) TRAC antigen sequence
AQKVTQAQSSVSMPVRKAVTLNCLYETSWWSYYIFWYKQLPSKEMIFLIRQGSDEQNAKSGRYSVNFKKAAKSVALTISALQLEDSAKYFCALGESLTRADKLIFGKGTRVTVEPNIQNPDPAVYQLRDSKSSDKSVCLFTDFDSQTNVSQSKDSDVYITDKTVLDMRSMDFKSNSAVAWSNKSDFACANAFNNSIIPEDTFFPSPESSCTTAPSAQLKKKLQALKKKNAQLKWKLQALKKKLAQGSGHHHHHH

SEQ ID NO: 124 - protein, 12 aa, Artificial Sequence
  Optional scFv tag sequence (kappa sequence + His tag)
RTAAASAHHHHH

SEQ ID NO: 125 - protein, 37 aa, Artificial Sequence
  Optional scFv tag sequence (kappa sequence + His and FLAG tag)
RTAAASAHHHHHHKLDYKDHDGDYKDHDIDYKDDDDK

SEQ ID NO: 126 - protein, 13 aa, Artificial Sequence
  Optional scFv tag sequence (lambda sequence + His tag)
GQPAAASAHHHHH

SEQ ID NO: 127 - protein, 38 aa, Artificial Sequence
  Optional scFv tag sequence (lambda sequence + His and FLAG tag)
GQPAAASAHHHHHHKLDYKDHDGDYKDHDIDYKDDDDK

SEQ ID NO: 128 - protein, 254 aa, Homo sapiens
  Polymorphic variant of SEQ ID NO: 1
AQKVTQAQSSVSMPVRKAVTLNCLYETSWWSYYIFWYKQLPSKEMIFLIRQGSDEQNAKSGRYSVNFKKAVKSVALTISALQLEDSAKYFCALGESLTRADKLIFGKGTRVTVEPNIQNPDPAVYQLRDSKSSDKSVCLFTDFDSQTNVSQSKDSDVYITDKTVLDMRSMDFKSNSAVAWSNKSDFACANAFNNSIIPEDTFFPSPESSCTTAPSAQLKKKLQALKKKNAQLKWKLQALKKKLAQGSGHHHHHH

SEQ ID NO: 129 - protein, 665 aa, Homo sapiens
  AD3 (variant 1245_P02_G04 with RTVAAPS sequence instead of RTAAAPS in kappa constant domain)
DIQMTQSPPALSASVGDRVTITCRASQDINDWLAWYQHKPGKAPKLLIYDASSLESGVPSRFSGSGSGTEFTLTISSLQPDDFATYYCQQSYSTPQVTFGQGTRLEIKRTVAAPSVFIFPPSDEQLKSGTASVVCLLNNFYPREAKVQWKVDNALQSGNSQESVTEQDSKDSTYSLSSTLTLSKADYEKHKVYACEVTHQGLSSPVTKSFNRGECEVQLQQSGPGLVKPSQTLSLTCAISGDSVSSKSAAWNWIRQSPSRGLEWLGRTYYRSKWSTDYAASVKSRITINPDTSKNQLSLQLNSVTPEDTAVYYCARTWSGYVDVWGQGTLVTVSSASTKGPSVFPLAPSSKSTSGGTAALGCLVKDYFPEPVTVSWNSGALTSGVHTFPAVLQSSGLYSLSSVVTVPSSSLGTQTYICNVNHKPSNTKVDKKVEPKSCDKTHTCPPCPAPELLGGPSVFLFPPKPKDTLMISRTPEVTCVVVDVSHEDPEVKFNWYVDGVEVHNAKTKPREEQYNSTYRVVSVLTVLHQDWLNGKEYKCKVSNKALPAPIEKTISKAKGQPREPQVYTLPPSRDELTKNQVSLTCLVKGFYPSDIAVEWESNGQPENNYKTTPPVLDSDGSFFLYSKLTVDKSRWQQGNVFSCSVMHEALHNHYTQKSLSLSPGK

SEQ ID NO: 130 - protein, 665 aa, Homo sapiens
  AD4 (variant 1245_P02_G04 with RTVAAPS sequence instead of RTAAAPS in kappa constant domain)
DIQMTQSPPALSASVGDRVTITCRASQDINDWLAWYQHKPGKAPKLLIYDASSLESGVPSRFSGSGSGTEFTLTISSLQPDDFATYYCQQSYSTPQVTFGQGTRLEIKRTVAAPSVFIFPPSDEQLKSGTASVVCLLNNFYPREAKVQWKVDNALQSGNSQESVTEQDSKDSTYSLSSTLTLSKADYEKHKVYACEVTHQGLSSPVTKSFNRGECEVQLQQSGPGLVKPSQTLSLTCAISGDSVSSKSAAWNWIRQSPSRGLEWLGRTYYRSKWSTDYAASVKSRITINPDTSKNQLSLQLNSVTPEDTAVYYCARTWSGYVDVWGQGTLVTVSSASTKGPSVFPLAPSSKSTSGGTAALGCLVKDYFPEPVTVSWNSGALTSGVHTFPAVLQSSGLYSLSSVVTVPSSSLGTQTYICNVNHKPSNTKVDKKVEPKSCDKTHTCPPCPAPELAGAPSVFLFPPKPKDTLMISRTPEVTCVVVDVSHEDPEVKFNWYVDGVEVHNAKTKPREEQYNSTYRVVSVLTVLHQDWLNGKEYKCKVSNKALPAPIEKTISKAKGQPREPQVYTLPPSRDELTKNQVSLTCLVKGFYPSDIAVEWESNGQPENNYKTTPPVLDSDGSFFLYSKLTVDKSRWQQGNVFSCSVMHEALHNHYTQKSLSLSPGK

SEQ ID NO: 131 - protein, 108 aa, Homo sapiens
  AD3 and AD4 full light chain variable sequence
DIQMTQSPPALSASVGDRVTITCRASQDINDWLAWYQHKPGKAPKLLIYDASSLESGVPSRFSGSGSGTEFTLTISSLQPDDFATYYCQQSYSTPQVTFGQGTRLEIK

SEQ ID NO: 132 - protein, 120 aa, Homo sapiens
  AD3 and AD4 full heavy chain variable sequence
EVQLQQSGPGLVKPSQTLSLTCAISGDSVSSKSAAWNWIRQSPSRGLEWLGRTYYRSKWSTDYAASVKSRITINPDTSKNQLSLQLNSVTPEDTAVYYCARTWSGYVDVWGQGTLVTVSS

SEQ ID NO: 133 - protein, 107 aa, Homo sapiens [sequence omitted]

SEQ ID NO: 134 - protein, 330 aa, Homo sapiens [sequence omitted]

SEQ ID NO: 135 - protein, 330 aa, Homo sapiens
  AD4 full heavy constant domain chain employed (with L235A, G237A modification)
ASTKGPSVFPLAPSSKSTSGGTAALGCLVKDYFPEPVTVSWNSGALTSGVHTFPAVLQSSGLYSLSSVVTVPSSSLGTQTYICNVNHKPSNTKVDKKVEPKSCDKTHTCPPCPAPELAGAPSVFLFPPKPKDTLMISRTPEVTCVVVDVSHEDPEVKFNWYVDGVEVHNAKTKPREEQYNSTYRVVSVLTVLHQDWLNGKEYKCKVSNKALPAPIEKTISKAKGQPREPQVYTLPPSRDELTKNQVSLTCLVKGFYPSDIAVEWESNGQPENNYKTTPPVLDSDGSFFLYSKLTVDKSRWQQGNVFSCSVMHEALHNHYTQKSLSLSPGK

SEQ ID NO: 136 - protein, 667 aa, Homo sapiens
  1245_P02_G04 with L235A, G237A) (aka G04 LAGA)
ASDIQMTQSPPALSASVGDRVTITCRASQDINDWLAWYQHKPGKAPKLLIYDASSLESGVPSRFSGSGSGTEFTLTISSLQPDDFATYYCQQSYSTPQVTFGQGTRLEIKRTAAAPSVFIFPPSDEQLKSGTASVVCLLNNFYPREAKVQWKVDNALQSGNSQESVTEQDSKDSTYSLSSTLTLSKADYEKHKLYACEVTHQGLSSPVTKSFNRGECQVQLQQSGPGLVKPSQTLSLTCAISGDSVSSKSAAWNWIRQSPSRGLEWLGRTYYRSKWSTDYAASVKSRITINPDTSKNQLSLQLNSVTPEDTAVYYCARTWSGYVDVWGQGTLVTVSSASTKGPSVFPLAPSSKSTSGGTAALGCLVKDYFPEPVTVSWNSGALTSGVHTFPAVLQSSGLYSLSSVVTVPSSSLGTQTYICNVNHKPSNTKVDKKVEPKSCDKTHTCPPCPAPELAGAPSVFLFPPKPKDTLMISRTPEVTCVVVDVSHEDPEVKFNWYVDGVEVHNAKTKPREEQYNSTYRVVSVLTVLHQDWLNGKEYKCKVSNKALPAPIEKTISKAKGQPREPQVYTLPPSRDELTKNQVSLTCLVKGFYPSDIAVEWESNGQPENNYKTTPPVLDSDGSFFLYSKLTVDKSRWQQGNVFSCSVMHEALHNHYTQKSLSLSPGK

SEQ ID NO: 137 - protein, 664 aa, Homo sapiens
  1245_P01_E07 with L235A, G237A (aka E07 LAGA)
ASDIQMTQSPSSLSASVGDRVTIACRAGQSIGTYLNWYQQKPGKAPKLLIYVASSLQSGVPSRFSGSGSGTEFTLTISSLQPEDFATYYCQQSYSTLLTFGRGTKVEIKRTAAAPSVFIFPPSDEQLKSGTASVVCLLNNFYPREAKVQWKVDNALQSGNSQESVTEQDSKDSTYSLSSTLTLSKADYEKHKLYACEVTHQGLSSPVTKSFNRGECQVQLVESGGGLVKPGGSLRLSCAASGFTFSDYYMSWIRQAPGKGLEWVSYISSSGSTIYYADSVKGRFTISRDNAKNSLYLQMNSLRAEDTAVYYCARVDYADAFDIWGQGTLVTVSSASTKGPSVFPLAPSSKSTSGGTAALGCLVKDYFPEPVTVSWNSGALTSGVHTFPAVLQSSGLYSLSSVVTVPSSSLGTQTYICNVNHKPSNTKVDKKVEPKSCDKTHTCPPCPAPELAGAPSVFLFPPKPKDTLMISRTPEVTCVVVDVSHEDPEVKFNWYVDGVEVHNAKTKPREEQYNSTYRVVSVLTVLHQDWLNGKEYKCKVSNKALPAPIEKTISKAKGQPREPQVYTLPPSRDELTKNQVSLTCLVKGFYPSDIAVEWESNGQPENNYKTTPPVLDSDGSFFLYSKLTVDKSRWQQGNVFSCSVMHEALHNHYTQKSLSLSPGK

SEQ ID NO: 138 - protein, 663 aa, Homo sapiens
  1252_P01_C08 with L235A, G237A (aka C08 LAGA)
ASSYELTQPPSVSVAPGKTARITCGGNNIGSQSVHWYQQKPGQAPMLVIYYDSDRPSGIPERFSGSNSGNTATLTISRVEAGDEADYYCQVWDSSSDHVVFGGGTKLTVLGQPAAAPSVTLFPPSSEELQANKATLVCLISDFYPGAVTVAWKADSSPVKAGVETTTPSKQSNNKYAASSYLSLTPEQWKSHRSYSCQVTHEGSTVEKTVAPTECSEVQLLESGGGLVQPGRSLRLSCAASGFTVSSNYMSWVRQAPGKGLEWVSVIYSGGSTYYADSVKGRFTISRDNSKNTLYLQMNSLRAEDTAVYYCASPIELGAFDIWGQGTLVTVSSASTKGPSVFPLAPSSKSTSGGTAALGCLVKDYFPEPVTVSWNSGALTSGVHTFPAVLQSSGLYSLSSVVTVPSSSLGTQTYICNVNHKPSNTKVDKKVEPKSCDKTHTCPPCPAPELAGAPSVFLFPPKPKDTLMISRTPEVTCVVVDVSHEDPEVKFNWYVDGVEVHNAKTKPREEQYNSTYRVVSVLTVLHQDWLNGKEYKCKVSNKALPAPIEKTISKAKGQPREPQVYTLPPSRDELTKNQVSLTCLVKGFYPSDIAVEWESNGQPENNYKTTPPVLDSDGSFFLYSKLTVDKSRWQQGNVFSCSVMHEALHNHYTQKSLSLSPGK

SEQ ID NO: 139 - protein, 661 aa, Homo sapiens
  D1.3 VH/VL + EGFR CH1/CH2/CH3 (LAGA)
ASDIQMTQSPSSLSASVGDRVTITCRASGNIHNYLAWYQQKPGKAPKLLIYYTTTLADGVPSRFSGSGSGTDYTFTISSLQPEDIATYYCQHFWSTPRTFGQGTKVEIKRTAAAPSVFIFPPSDEQLKSGTASVVCLLNNFYPREAKVQWKVDNALQSGNSQESVTEQDSKDSTYSLSSTLTLSKADYEKHKLYACEVTHQGLSSPVTKSFNRGECQVQLQESGPGLVRPSQTLSLTCTVSGSTFSGYGVNWVRQPPGRGLEWIGMIWGDGNTDYNSALKSRVTMLVDTSKNQFSLRLSSVTAADTAVYYCARERDYRLDYWGQGSLVTVSSASTKGPSVFPLAPSSKSTSGGTAALGCLVKDYFPEPVTVSWNSGALTSGVHTFPAVLQSSGLYSLSSVVTVPSSSLGTQTYICNVNHKPSNTKVDKKVEPKSCDKTHTCPPCPAPELAGAPSVFLFPPKPKDTLMISRTPEVTCVVVDVSHEDPEVKFNWYVDGVEVHNAKTKPREEQYNSTYRVVSVLTVLHQDWLNGKEYKCKVSNKALPAPIEKTISKAKGQPREPQVYTLPPSRDETDDGPVSLTCLVKGFYPSDIAVEWESTYGPENNYKTTPPVLDSDGSFFLYSKLTVSYWRWYKGNVFSCSVMHEALHNHYTQKSLSLSPG

SEQ ID NO: 140 - protein, 662 aa, Homo sapiens
  1252_P01_C08 VH/VL + CH1/CH2/CH3 EGFR (LAGA)
ASSYELTQPPSVSVAPGKTARITCGGNNIGSQSVHWYQQKPGQAPMLVIYYDSDRPSGIPERFSGSNSGNTATLTISRVEAGDEADYYCQVWDSSSDHVVFGGGTKLTVLGQPAAAPSVTLFPPSSEELQANKATLVCLISDFYPGAVTVAWKADSSPVKAGVETTTPSKQSNNKYAASSYLSLTPEQWKSHRSYSCQVTHEGSTVEKTVAPTECSEVQLLESGGGLVQPGRSLRLSCAASGFTVSSNYMSWVRQAPGKGLEWVSVIYSGGSTYYADSVKGRFTISRDNSKNTLYLQMNSLRAEDTAVYYCASPIELGAFDIWGQGTLVTVSSASTKGPSVFPLAPSSKSTSGGTAALGCLVKDYFPEPVTVSWNSGALTSGVHTFPAVLQSSGLYSLSSVVTVPSSSLGTQTYICNVNHKPSNTKVDKKVEPKSCDKTHTCPPCPAPELAGAPSVFLFPPKPKDTLMISRTPEVTCVVVDVSHEDPEVKFNWYVDGVEVHNAKTKPREEQYNSTYRVVSVLTVLHQDWLNGKEYKCKVSNKALPAPIEKTISKAKGQPREPQVYTLPPSRDETDDGPVSLTCLVKGFYPSDIAVEWESTYGPENNYKTTPPVLDSDGSFFLYSKLTVSYWRWYKGNVFSCSVMHEALHNHYTQKSLSLSPG

SEQ ID NO: 141 - protein, 666 aa, Homo sapiens
  1245_P02_G04 VH/VL + CH1/CH2/CH3 EGFR (LAGA)
ASDIQMTQSPPALSASVGDRVTITCRASQDINDWLAWYQHKPGKAPKLLIYDASSLESGVPSRFSGSGSGTEFTLTISSLQPDDFATYYCQQSYSTPQVTFGQGTRLEIKRTAAAPSVFIFPPSDEQLKSGTASVVCLLNNFYPREAKVQWKVDNALQSGNSQESVTEQDSKDSTYSLSSTLTLSKADYEKHKLYACEVTHQGLSSPVTKSFNRGECQVQLQQSGPGLVKPSQTLSLTCAISGDSVSSKSAAWNWIRQSPSRGLEWLGRTYYRSKWSTDYAASVKSRITINPDTSKNQLSLQLNSVTPEDTAVYYCARTWSGYVDVWGQGTLVTVSSASTKGPSVFPLAPSSKSTSGGTAALGCLVKDYFPEPVTVSWNSGALTSGVHTFPAVLQSSGLYSLSSVVTVPSSSLGTQTYICNVNHKPSNTKVDKKVEPKSCDKTHTCPPCPAPELAGAPSVFLFPPKPKDTLMISRTPEVTCVVVDVSHEDPEVKFNWYVDGVEVHNAKTKPREEQYNSTYRVVSVLTVLHQDWLNGKEYKCKVSNKALPAPIEKTISKAKGQPREPQVYTLPPSRDETDDGPVSLTCLVKGFYPSDIAVEWESTYGPENNYKTTPPVLDSDGSFFLYSKLTVSYWRWYKGNVFSCSVMHEALHNHYTQKSLSLSPG

SEQ ID NO: 142 - protein, 663 aa, Homo sapiens
  1245_P01_E07 VH/VL + CH1/CH2/CH3 EGFR (LAGA)
ASDIQMTQSPSSLSASVGDRVTIACRAGQSIGTYLNWYQQKPGKAPKLLIYVASSLQSGVPSRFSGSGSGTEFTLTISSLQPEDFATYYCQQSYSTLLTFGRGTKVEIKRTAAAPSVFIFPPSDEQLKSGTASVVCLLNNFYPREAKVQWKVDNALQSGNSQESVTEQDSKDSTYSLSSTLTLSKADYEKHKLYACEVTHQGLSSPVTKSFNRGECQVQLVESGGGLVKPGGSLRLSCAASGFTFSDYYMSWIRQAPGKGLEWVSYISSSGSTIYYADSVKGRFTISRDNAKNSLYLQMNSLRAEDTAVYYCARVDYADAFDIWGQGTLVTVSSASTKGPSVFPLAPSSKSTSGGTAALGCLVKDYFPEPVTVSWNSGALTSGVHTFPAVLQSSGLYSLSSVVTVPSSSLGTQTYICNVNHKPSNTKVDKKVEPKSCDKTHTCPPCPAPELAGAPSVFLFPPKPKDTLMISRTPEVTCVVVDVSHEDPEVKFNWYVDGVEVHNAKTKPREEQYNSTYRVVSVLTVLHQDWLNGKEYKCKVSNKALPAPIEKTISKAKGQPREPQVYTLPPSRDETDDGPVSLTCLVKGFYPSDIAVEWESTYGPENNYKTTPPVLDSDGSFFLYSKLTVSYWRWYKGNVFSCSVMHEALHNHYTQKSLSLSPG

SEQ ID NO: 143 - protein, 917 aa, Homo sapiens
  D1.3 LAGA + scFV (derived from Cetuximab)
ASDIQMTQSPSSLSASVGDRVTITCRASGNIHNYLAWYQQKPGKAPKLLIYYTTTLADGVPSRFSGSGSGTDYTFTISSLQPEDIATYYCQHFWSTPRTFGQGTKVEIKRTAAAPSVFIFPPSDEQLKSGTASVVCLLNNFYPREAKVQWKVDNALQSGNSQESVTEQDSKDSTYSLSSTLTLSKADYEKHKLYACEVTHQGLSSPVTKSFNRGECQVQLQESGPGLVRPSQTLSLTCTVSGSTFSGYGVNWVRQPPGRGLEWIGMIWGDGNTDYNSALKSRVTMLVDTSKNQFSLRLSSVTAADTAVYYCARERDYRLDYWGQGSLVTVSSASTKGPSVFPLAPSSKSTSGGTAALGCLVKDYFPEPVTVSWNSGALTSGVHTFPAVLQSSGLYSLSSVVTVPSSSLGTQTYICNVNHKPSNTKVDKKVEPKSCDKTHTCPPCPAPELAGAPSVFLFPPKPKDTLMISRTPEVTCVVVDVSHEDPEVKFNWYVDGVEVHNAKTKPREEQYNSTYRVVSVLTVLHQDWLNGKEYKCKVSNKALPAPIEKTISKAKGQPREPQVYTLPPSRDELTKNQVSLTCLVKGFYPSDIAVEWESNGQPENNYKTTPPVLDSDGSFFLYSKLTVDKSRWQQGNVFSCSVMHEALHNHYTQKSLSLSPGGGGGSGGGGSGGGGSQVQLKQSGPGLVQPSQSLSITCTVSGFSLTNYGVHWVRQSPGKGLEWLGVIWSGGNTDYNTPFTSRLSINKDNSKSQVFFKMNSLQSNDTAIYYCARALTYYDYEFAYWGQGTLVTVSAGGGGSGGGGSGGGGSDILLTQSPVILSVSPGERVSFSCRASQSIGTNIHWYQQRTNGSPRLLIKYASESISGIPSRFSGSGSGTDFTLSINSVESEDIADYYCQQNNNWPTTFGAGTKLELK

SEQ ID NO: 144 - protein, 918 aa, Homo sapiens
  C08 LAGA + scFV (derived from Cetuximab)
ASSYELTQPPSVSVAPGKTARITCGGNNIGSQSVHWYQQKPGQAPMLVIYYDSDRPSGIPERFSGSNSGNTATLTISRVEAGDEADYYCQVWDSSSDHVVFGGGTKLTVLGQPAAAPSVTLFPPSSEELQANKATLVCLISDFYPGAVTVAWKADSSPVKAGVETTTPSKQSNNKYAASSYLSLTPEQWKSHRSYSCQVTHEGSTVEKTVAPTECSEVQLLESGGGLVQPGRSLRLSCAASGFTVSSNYMSWVRQAPGKGLEWVSVIYSGGSTYYADSVKGRFTISRDNSKNTLYLQMNSLRAEDTAVYYCASPIELGAFDIWGQGTLVTVSSASTKGPSVFPLAPSSKSTSGGTAALGCLVKDYFPEPVTVSWNSGALTSGVHTFPAVLQSSGLYSLSSVVTVPSSSLGTQTYICNVNHKPSNTKVDKKVEPKSCDKTHTCPPCPAPELAGAPSVFLFPPKPKDTLMISRTPEVTCVVVDVSHEDPEVKFNWYVDGVEVHNAKTKPREEQYNSTYRVVSVLTVLHQDWLNGKEYKCKVSNKALPAPIEKTISKAKGQPREPQVYTLPPSRDELTKNQVSLTCLVKGFYPSDIAVEWESNGQPENNYKTTPPVLDSDGSFFLYSKLTVDKSRWQQGNVFSCSVMHEALHNHYTQKSLSLSPGGGGGSGGGGSGGGGSQVQLKQSGPGLVQPSQSLSITCTVSGFSLTNYGVHWVRQSPGKGLEWLGVIWSGGNTDYNTPFTSRLSINKDNSKSQVFFKMNSLQSNDTAIYYCARALTYYDYEFAYWGQGTLVTVSAGGGGSGGGGSGGGGSDILLTQSPVILSVSPGERVSFSCRASQSIGTNIHWYQQRTNGSPRLLIKYASESISGIPSRFSGSGSGTDFTLSINSVESEDIADYYCQQNNNWPTTFGAGTKLELK

SEQ ID NO: 145 - protein, 922 aa, Homo sapiens
  G04 LAGA + scFV (derived from Cetuximab)
ASDIQMTQSPPALSASVGDRVTITCRASQDINDWLAWYQHKPGKAPKLLIYDASSLESGVPSRFSGSGSGTEFTLTISSLQPDDFATYYCQQSYSTPQVTFGQGTRLEIKRTAAAPSVFIFPPSDEQLKSGTASVVCLLNNFYPREAKVQWKVDNALQSGNSQESVTEQDSKDSTYSLSSTLTLSKADYEKHKLYACEVTHQGLSSPVTKSFNRGECQVQLQQSGPGLVKPSQTLSLTCAISGDSVSSKSAAWNWIRQSPSRGLEWLGRTYYRSKWSTDYAASVKSRITINPDTSKNQLSLQLNSVTPEDTAVYYCARTWSGYVDVWGQGTLVTVSSASTKGPSVFPLAPSSKSTSGGTAALGCLVKDYFPEPVTVSWNSGALTSGVHTFPAVLQSSGLYSLSSVVTVPSSSLGTQTYICNVNHKPSNTKVDKKVEPKSCDKTHTCPPCPAPELAGAPSVFLFPPKPKDTLMISRTPEVTCVVVDVSHEDPEVKFNWYVDGVEVHNAKTKPREEQYNSTYRVVSVLTVLHQDWLNGKEYKCKVSNKALPAPIEKTISKAKGQPREPQVYTLPPSRDELTKNQVSLTCLVKGFYPSDIAVEWESNGQPENNYKTTPPVLDSDGSFFLYSKLTVDKSRWQQGNVFSCSVMHEALHNHYTQKSLSLSPGGGGGSGGGGSGGGGSQVQLKQSGPGLVQPSQSLSITCTVSGFSLTNYGVHWVRQSPGKGLEWLGVIWSGGNTDYNTPFTSRLSINKDNSKSQVFFKMNSLQSNDTAIYYCARALTYYDYEFAYWGQGTLVTVSAGGGGSGGGGSGGGGSDILLTQSPVILSVSPGERVSFSCRASQSIGTNIHWYQQRTNGSPRLLIKYASESISGIPSRFSGSGSGTDFTLSINSVESEDIADYYCQQNNNWPTTFGAGTKLELK

SEQ ID NO: 146 - protein, 919 aa, Homo sapiens
  E07 LAGA + scFV (derived from Cetuximab)
ASDIQMTQSPSSLSASVGDRVTIACRAGQSIGTYLNWYQQKPGKAPKLLIYVASSLQSGVPSRFSGSGSGTEFTLTISSLQPEDFATYYCQQSYSTLLTFGRGTKVEIKRTAAAPSVFIFPPSDEQLKSGTASVVCLLNNFYPREAKVQWKVDNALQSGNSQESVTEQDSKDSTYSLSSTLTLSKADYEKHKLYACEVTHQGLSSPVTKSFNRGECQVQLVESGGGLVKPGGSLRLSCAASGFTFSDYYMSWIRQAPGKGLEWVSYISSSGSTIYYADSVKGRFTISRDNAKNSLYLQMNSLRAEDTAVYYCARVDYADAFDIWGQGTLVTVSSASTKGPSVFPLAPSSKSTSGGTAALGCLVKDYFPEPVTVSWNSGALTSGVHTFPAVLQSSGLYSLSSVVTVPSSSLGTQTYICNVNHKPSNTKVDKKVEPKSCDKTHTCPPCPAPELAGAPSVFLFPPKPKDTLMISRTPEVTCVVVDVSHEDPEVKFNWYVDGVEVHNAKTKPREEQYNSTYRVVSVLTVLHQDWLNGKEYKCKVSNKALPAPIEKTISKAKGQPREPQVYTLPPSRDELTKNQVSLTCLVKGFYPSDIAVEWESNGQPENNYKTTPPVLDSDGSFFLYSKLTVDKSRWQQGNVFSCSVMHEALHNHYTQKSLSLSPGGGGGSGGGGSGGGGSQVQLKQSGPGLVQPSQSLSITCTVSGFSLTNYGVHWVRQSPGKGLEWLGVIWSGGNTDYNTPFTSRLSINKDNSKSQVFFKMNSLQSNDTAIYYCARALTYYDYEFAYWGQGTLVTVSAGGGGSGGGGSGGGGSDILLTQSPVILSVSPGERVSFSCRASQSIGTNIHWYQQRTNGSPRLLIKYASESISGIPSRFSGSGSGTDFTLSINSVESEDIADYYCQQNNNWPTTFGAGTKLELK

SEQ ID NO: 147 - protein, 329 aa, Homo sapiens
  CH1-CH2-CH3 EGFR binding module
ASTKGPSVFPLAPSSKSTSGGTAALGCLVKDYFPEPVTVSWNSGALTSGVHTFPAVLQSSGLYSLSSVVTVPSSSLGTQTYICNVNHKPSNTKVDKKVEPKSCDKTHTCPPCPAPELLGGPSVFLFPPKPKDTLMISRTPEVTCVVVDVSHEDPEVKFNWYVDGVEVHNAKTKPREEQYNSTYRVVSVLTVLHQDWLNGKEYKCKVSNKALPAPIEKTISKAKGQPREPQVYTLPPSRDETDDGPVSLTCLVKGFYPSDIAVEWESTYGPENNYKTTPPVLDSDGSFFLYSKLTVSYWRWYKGNVFSCSVMHEALHNHYTQKSLSLSPG

SEQ ID NO: 148 - protein, 329 aa, Homo sapiens
  CH1-CH2-CH3 EGFR binding module (with LAGA)
ASTKGPSVFPLAPSSKSTSGGTAALGCLVKDYFPEPVTVSWNSGALTSGVHTFPAVLQSSGLYSLSSVVTVPSSSLGTQTYICNVNHKPSNTKVDKKVEPKSCDKTHTCPPCPAPELAGAPSVFLFPPKPKDTLMISRTPEVTCVVVDVSHEDPEVKFNWYVDGVEVHNAKTKPREEQYNSTYRVVSVLTVLHQDWLNGKEYKCKVSNKALPAPIEKTISKAKGQPREPQVYTLPPSRDETDDGPVSLTCLVKGFYPSDIAVEWESTYGPENNYKTTPPVLDSDGSFFLYSKLTVSYWRWYKGNVFSCSVMHEALHNHYTQKSLSLSPG

SEQ ID NO: 149 - protein, 241 aa, Homo sapiens
  scFv (Cetuximab derived) binding module
QVQLKQSGPGLVQPSQSLSITCTVSGFSLTNYGVHWVRQSPGKGLEWLGVIWSGGNTDYNTPFTSRLSINKDNSKSQVFFKMNSLQSNDTAIYYCARALTYYDYEFAYWGQGTLVTVSAGGGGSGGGGSGGGGSDILLTQSPVILSVSPGERVSFSCRASQSIGTNIHWYQQRTNGSPRLLIKYASESISGIPSRFSGSGSGTDFTLSINSVESEDIADYYCQQNNNWPTTFGAGTKLELK

SEQ ID NO: 150 - protein, 20 aa, Homo sapiens
  N-terminal leader sequence of the V delta 1 chain
MLFSSLLCVFVAFSYSGSSV

SEQ ID NO: 151 - protein, 95 aa, Homo sapiens
  V region of the V delta 1 chain
AQKVTQAQSSVSMPVRKAVTLNCLYETSWWSYYIFWYKQLPSKEMIFLIRQGSDEQNAKSGRYSVNFKKAAKSVALTISALQLEDSAKYFCALGE

SEQ ID NO: 152 - protein, 16 aa, Homo sapiens
  J1*0 - one of the four J regions encoded in the human delta one chain germline
TDKLIFGKGTRVTVEP

SEQ ID NO: 153 - protein, 17 aa, Homo sapiens
  J2*0 - one of the four J regions encoded in the human delta one chain germline
LTAQLFFGKGTQLIVEP

SEQ ID NO: 154 - protein, 19 aa, Homo sapiens
  J3*0 - one of the four J regions encoded in the human delta one chain germline
SWDTRQMFFGTGIKLFVEP

SEQ ID NO: 155 - protein, 15 aa, Homo sapiens
  J4*0 - one of the four J regions encoded in the human delta one chain germline
RPLIFGKGTYLEVQQ

SEQ ID NO: 156 - protein, 153 aa, Homo sapiens
  C1*0 C-region of the V delta 1 chain
  misc_feature (1)..(1): Xaa can be any naturally occurring amino acid
XSQPHTKPSVFVMKNGTNVACLVKEFYPKDIRINLVSSKKITEFDPAIVISPSGKYNAVKLGKYESNSVTCSVQHDNKTVHSTDFEVKTDSTDHVKPKETENTKQPSKSCHKPKAIVHTEKVNMMSLTVLGLRMLFAKTVAVNFLLTAKLFFL

SEQ ID NO: 157 - protein, 250 aa, Homo sapiens
  scFv anti-CD19 binding module
QVQLQQSGAELVRPGSSVKISCKASGYAFSSYWMNWVKQRPGQGLEWIGQIWPGDGDTNYNGKFKGKATLTADESSSTAYMQLSSLASEDSAVYFCARRETTTVGRYYYAMDYWGQGTTVTVSSGGGGSGGGGSGGGGSDIQLTQSPASLAVSLGQRATISCKASQSVDYDGDSYLNWYQQIPGQPPKLLIYDASNLVSGIPPRFSGSGSGTDFTLNIHPVEKVDAATYHCQQSTEDPWTFGGGTKLEIK

SEQ ID NO: 158 - protein, 931 aa, Homo sapiens
  G04 x Anti-CD19 multispecific (full length)
ASDIQMTQSPPALSASVGDRVTITCRASQDINDWLAWYQHKPGKAPKLLIYDASSLESGVPSRFSGSGSGTEFTLTISSLQPDDFATYYCQQSYSTPQVTFGQGTRLEIKRTAAAPSVFIFPPSDEQLKSGTASVVCLLNNFYPREAKVQWKVDNALQSGNSQESVTEQDSKDSTYSLSSTLTLSKADYEKHKLYACEVTHQGLSSPVTKSFNRGECQVQLQQSGPGLVKPSQTLSLTCAISGDSVSSKSAAWNWIRQSPSRGLEWLGRTYYRSKWSTDYAASVKSRITINPDTSKNQLSLQLNSVTPEDTAVYYCARTWSGYVDVWGQGTLVTVSSASTKGPSVFPLAPSSKSTSGGTAALGCLVKDYFPEPVTVSWNSGALTSGVHTFPAVLQSSGLYSLSSVVTVPSSSLGTQTYICNVNHKPSNTKVDKKVEPKSCDKTHTCPPCPAPELAGAPSVFLFPPKPKDTLMISRTPEVTCVVVDVSHEDPEVKFNWYVDGVEVHNAKTKPREEQYNSTYRVVSVLTVLHQDWLNGKEYKCKVSNKALPAPIEKTISKAKGQPREPQVYTLPPSRDELTKNQVSLTCLVKGFYPSDIAVEWESNGQPENNYKTTPPVLDSDGSFFLYSKLTVDKSRWQQGNVFSCSVMHEALHNHYTQKSLSLSPGGGGGSGGGGSGGGGSQVQLQQSGAELVRPGSSVKISCKASGYAFSSYWMNWVKQRPGQGLEWIGQIWPGDGDTNYNGKFKGKATLTADESSSTAYMQLSSLASEDSAVYFCARRETTTVGRYYYAMDYWGQGTTVTVSSGGGGSGGGGSGGGGSDIQLTQSPASLAVSLGQRATISCKASQSVDYDGDSYLNWYQQIPGQPPKLLIYDASNLVSGIPPRFSGSGSGTDFTLNIHPVEKVDAATYHCQQSTEDPWTFGGGTKLEIK

SEQ ID NO: 159 - protein, 928 aa, Homo sapiens
  E07 x Anti-CD19 multispecific (full length)
ASDIQMTQSPSSLSASVGDRVTIACRAGQSIGTYLNWYQQKPGKAPKLLIYVASSLQSGVPSRFSGSGSGTEFTLTISSLQPEDFATYYCQQSYSTLLTFGRGTKVEIKRTAAAPSVFIFPPSDEQLKSGTASVVCLLNNFYPREAKVQWKVDNALQSGNSQESVTEQDSKDSTYSLSSTLTLSKADYEKHKLYACEVTHQGLSSPVTKSFNRGECQVQLVESGGGLVKPGGSLRLSCAASGFTFSDYYMSWIRQAPGKGLEWVSYISSSGSTIYYADSVKGRFTISRDNAKNSLYLQMNSLRAEDTAVYYCARVDYADAFDIWGQGTLVTVSSASTKGPSVFPLAPSSKSTSGGTAALGCLVKDYFPEPVTVSWNSGALTSGVHTFPAVLQSSGLYSLSSVVTVPSSSLGTQTYICNVNHKPSNTKVDKKVEPKSCDKTHTCPPCPAPELAGAPSVFLFPPKPKDTLMISRTPEVTCVVVDVSHEDPEVKFNWYVDGVEVHNAKTKPREEQYNSTYRVVSVLTVLHQDWLNGKEYKCKVSNKALPAPIEKTISKAKGQPREPQVYTLPPSRDELTKNQVSLTCLVKGFYPSDIAVEWESNGQPENNYKTTPPVLDSDGSFFLYSKLTVDKSRWQQGNVFSCSVMHEALHNHYTQKSLSLSPGGGGGSGGGGSGGGGSQVQLQQSGAELVRPGSSVKISCKASGYAFSSYWMNWVKQRPGQGLEWIGQIWPGDGDTNYNGKFKGKATLTADESSSTAYMQLSSLASEDSAVYFCARRETTTVGRYYYAMDYWGQGTTVTVSSGGGGSGGGGSGGGGSDIQLTQSPASLAVSLGQRATISCKASQSVDYDGDSYLNWYQQIPGQPPKLLIYDASNLVSGIPPRFSGSGSGTDFTLNIHPVEKVDAATYHCQQSTEDPWTFGGGTKLEIK

SEQ ID NO: 160 - protein, 3 aa, Homo sapiens
  E07 Light CDR2
VAS

SEQ ID NO: 161 - protein, 3 aa, Homo Sapiens
  C08 Light CDR2
YDS

SEQ ID NO: 162 - protein, 3 aa, Homo Sapiens
  G04 Light CDR2
DAS

SEQ ID NO: 163 - protein, 3 aa, Homo Sapiens
  B07 Light CDR2
AAS

SEQ ID NO: 164 - protein, 3 aa, Homo Sapiens
  C05 Light CDR2
DAS

SEQ ID NO: 165 - protein, 3 aa, Homo Sapiens
  E01 Light CDR2
EVS

SEQ ID NO: 166 - protein, 3 aa, Homo Sapiens
  E04 Light CDR2
DAS

SEQ ID NO: 167 - protein, 3 aa, Homo Sapiens
  F07 Light CDR2
DAS

SEQ ID NO: 168 - protein, 3 aa, Homo Sapiens
  G06 Light CDR2
AAS

SEQ ID NO: 169 - protein, 3 aa, Homo Sapiens
  G09 Light CDR2
DAS

SEQ ID NO: 170 - protein, 3 aa, Homo Sapiens
  B09 Light CDR2
DAS

SEQ ID NO: 171 - protein, 3 aa, Homo Sapiens
  G10 Light CDR2
AAS

SEQ ID NO: 172 - protein, 92 aa, Homo Sapiens
  Cyno variable delta 1 (V delta 1) chain of a gamma delta T cell receptor (TCR) - aka cyno TRDV1
AQKVTQAQSSVSMPVEKAVTLNCQYETSSWSYDLFWYKQLPGKEMIFLIHQGSSQQNARNGRYSVNFQKAASSITLTISALQLEDSATYFCA

SEQ ID NO: 173 - protein, 101 aa, Homo Sapiens
  Human variable delta 4 chain of a gamma delta T cell receptor (TCR) - aka human TRGV4
KSSNLEGRTKSVIRQTGSSAEITCDLAEGSTGYIHWYLHQEGKAPQRLLYYDSYTSSVVLESGISPGKYDTYGSTRKNLRMILRNLIENDSGVYYCATWDG

SEQ ID NO: 174 - protein, 96 aa, Homo Sapiens
  Human variable delta 2 (V delta 2) chain of a gamma delta T cell receptor (TCR) - aka TRDV2
AIELVPEHQTVPVSIGVPATLRCSMKGEAIGNYYINWYRKTQGNTMTFIYREKDIYGPGFKDNFQGDIDIAKNLAVLKILAPSERDEGSYYCACDT

SEQ ID NO: 175 - protein, 95 aa, Homo Sapiens
  Human variable delta 3 (V delta 3) chain of a gamma delta T cell receptor (TCR) - aka TRDV3
DKVTQSSPDQTVASGSEVVLLCTYDTVYSNPDLFWYRIRPDYSFQFVFYGDNSRSEGADFTQGRFSVKHILTQKAFHLVISPVRTEDSATYYCAF

SEQ ID NO: 176 - protein, 257 aa, Homo sapiens
  Folate receptor alpha
MAQRMTTQLLLLLVWVAVVGEAQTRIAWARTELLNVCMNAKHHKEKPGPEDKLHEQCRPWRKNACCSTNTSQEAHKDVSYLYRFNWNHCGEMAPACKRHFIQDTCLYECSPNLGPWIQQVDQSWRKERVLNVPLCKEDCEQWWEDCRTSYTCKSNWHKGWNWTSGFNKCAVGAACQPFHFYFPTPTVLCNEIWTHSYKVSNYSRGSGRCIQMWFDPAQGNPNEEVARFYAAAMSGAGPWAAWPFLLSLALMLLWLLS